European Patent Application EP 4 477 226 A1, published December 18, 2024. Title: COMPOSITIONS COMPRISING RECOMBINANT MYCOBACTERIUM STRAINS, USES AND METHODS FOR THE PREVENTION AND/OR TREATMENT OF CANCER THEREOF. Applicant: INSTITUTO BUTANTAN. The sequence listing filed with the application follows.

SEQUENCE LISTING (3 sequences)

SEQ ID NO: 1 - DNA, 32 bp, synthetic construct
  misc_feature 1..32: note = N-terminal primer for the LTK63 gene
  source 1..32: mol_type = other DNA
tagggatccaatggcgacagattataccgttg

SEQ ID NO: 2 - DNA, 33 bp, synthetic construct
  misc_feature 1..33: note = C-terminal primer for the LTK63 gene
  source 1..33: mol_type = other DNA
tagggtacctaattcatcccgaattctgttata

SEQ ID NO: 3 - DNA, 7488 bp, synthetic construct
  misc_feature 1..7488: note = Plasm deo pNL12-LTAK63
  source 1..7488: mol_type = other DNA
gcgcccaatacgcaaaccgcctctccccgcgcgttggccgattcattaatgcagctggcacgacaggtttcccgactggaaagcgggcagtgagcgcaacgcaattaatgtgagttagctcactcattaggcaccccaggctttacactttatgcttccggctcgtatgttgtgtggaattgtgagcggataacaatttcacacaggaaacagctatgaccatgattacgaattcgagctcgacttaattaactccgggtggtcactgagtacatcccgtcggtgcgttcggcatcggtcggggtgtgggtgggtgtcggctcccgcgacgaaggacgaagcgtcgcgggtgccgcccacttcttggagcatctgctgttcaaggccaccccgacgcgcacgcggtcgacatcgcgcaggctgtcgatgccgtcggcggtgagctgaacgcgttcaccacgcgcgagcacacctgttactacgcgcatgtgctcgactccgacctggagctcgcggtcgacctggtgcgccgatgtcgtgttgcgtgggcgttgtgccaccgaggatgtcgaagtggagcgcgacgtcgtcctcgaggagatcgccatgcgtgacgacgatcccgaggacagcctcggcgacgtgttcctctcggcgatgttcggcgatcacccggtgggacgtccggtgatcggcagcgtcgagtcgatcgagaccatgacgcgtgcacagctgcattcgttccacgtccggcgttacacacccgaacggatgatcgtggcggtggccggcaacgtcgaccacgacgtgtggtgtcgttggtccgagagcatttcggcccccggctggaggccgacgttccgcggtggctccccgtaaggctcgggacgggtcggtggtaagccatcgctgctcgtggtcgaccgcgacggggaacagtcccatgtctcgctgggcgttcgcacgcccggccggcactgggagcaccggtgggccctgtcggtgttgaacaccgcgctgggaggcgggctcagttctcgtctgttccaacagattcgcgagtcccgcggcctggcctacctcggtgtactcgaccgtggaccacttcgcgacagcggggctctgtcggtgtatgcgggatgtcagccggaacgtttcgacgaagtggtgcgggtgaccaccgaagttttggaaggtgttgccagagacgggatcaccgccgacgaatgccggatcgccaaaggctcgttgcgcggtgggctggtgctcggcctggaggattccggatcacgtatgcaccggatcggccgtagcgagctcaattacggtggagcaccggaccatcgaccacacgctggcccagatcgaggcagtcactctagaagaggtcaacgccgtcgctcaccagttgctgtcgcgggactacggtgccgccgtactcggtccctatagttcgaaaaaggcgctgccacaacagcttcaaactatcgccggctgacccgctacactgggtccaatggattagaaggagaagtaccgatgggatccggtaccaatggcgacagattataccgtgctgactctagacccccagatgaaataaaacgttccggaggtcttatgcccagagggcataatgagtacttcgatagaggaactcaaatgaatattaatctttatgatcacgcgagaggaacacaaaccggctttgtcagatatgatgacggatatgtttccactaagcttagtttgagaagtgctcacttagcaggacagtctatattatcaggatattccacttactatatatatgttatagcgacagcaccaaatatgtttaatgttaatgatgtattaggcgtatacagccctcacccatatgaacaggaggtttctgcgttaggtggaataccatattctcagatatatggatggtatcgtgttaattttggtgtgattgatgaacgattacatcgtaacagggaatatagagaccggtattacagaaatctgaatatagctccggcagaggatggttacagattagcaggtttcccaccggatcaccaagcttggagagaagaaccctggattcatcatgcaccacaaggttgtggaaattcatcaagaacaatcacaggtgatacttgtaatgaggagacccagaatctgagcacaatatatctcagggaatatcaatcaaaagttaagaggcagatattttcagactatcagtcagaggttgacatatataacagaattcgggatgaattatgactgcagcatcaccatcaccatcactagtgaaatagcgaaacacgggatcgggcgagttcgaccttccgtcggtctcgccctattaatagtggcatgcaagcttggcactggccgtcgttttacaacgtcgtgactgggaaaaccctggcgttacccaacttaatcgccttgcagcacatccccctttcgccagctggcgtaatagcgaagaggcccgcaccgatcgcccttcccaacagttgcgcagcctgaatggcgaatggcgcctgatgcggtattttctccttacgcatctgtgcggtatttcacaccgcatatgcaggggggggggggcgctgaggtctgcctcgtgaagaaggtgttgctgactcataccaggaacgaggacagtcgcacgacgaagttcttctggatcgcgcccgtgctggaagcactcaacctcgaagcgtgtggttgcggagccatctagcaaccacacgaaacatgcgcaacgaaccgcgcaacgaacaacgcctagaactggccctagatgagctgactcgtatcgttggtaaacctagtttgaccagcatgttttaactacgttcggtgagctgtcaacggggcctgtaacggcacaacgaaccgtgcaacgagagtggccacggatgccaccacaggcactacaacggagttcgccacgtacatcaccacaaccaccgattctggcggtgagctccccgatattcagcggaaatggcttggtatcgaccaagattcgtagaaccccgtctcgtctggctggtattcaaaacgggcgcaacgaaacacgcaacgagacaggcatggcccaaaccagaaaactagcgtctaccaggacttttacctgtccgacccgttgcaacggaaccccccacggaacccccgcgacacccgctccccaattgcgttagaacagcggtggattgtcggcttcgttgtgggccttttgagccgcttcctgttctgccgcacgctctttcctcgcccgatagccgagtcgcttaacggtgtccagatgcagcccgaaatgtttggccgtttgcggccaagagtggccctcgtcgtcgtgataggcgcggatgcgttcgcggcgtgcagcctgctcggcgagccactcgctgcgttcctgcgccacgagccggacgacgtggcgttcggatagtccggtgattcgagcgccttcggcggcggtcacgcgccgctttttgcggacagtcggctgccggttgtagccgtcgctgtagccgtcgctcatagcaatgcctccatggctgacgcggactttgcgcgccgcgcaactgtgctcgccgccgtgcgcgctgctgcgcccttccgcgagatggccgactggcgcgcactgagtgtggcctcgtagaccacgatcccgtccgcccaaatgcgcgacttggttgtgatccaacgccaaatgctgttggcgatggcgcggacctcgctgtccggtagcggtccgggacacacgtcgttgcacgggaattcggcgtttcgcgcgtggcactcggcatagatcgcgcggccgagtccgtccacgttccgggtcggcaggtagatccgcatgagggcgggacgataggcccacaacctgacggaatcgaacagtgcgcaattccgccctagcggcgtcggagccgctttgtacgtggtctgctgacgccagcgcggcggtggcatgttcgcgccgagctcggcctcgatgtggctgagtgtgtagagatctgagtggagccattccgtttcccaggcgatgtggccggggtttttggtcatgaggcctgagtaactgcggtcgccgtcgacggcgcgccgaaggccttcggcgcacgccgccatgtatgcgagcggcttacgccgcgcgtattcggtgcgtggaacaggggcgttgagtgcccacactgcgtgtgcgtggccgttggcgcgattgcccacgatcgcgttgggcagcggatgggacccccgggcgctgagcgctcggagcgctgcgtctggatggtctacgtccacgaccagcaggtttgccagcgctgttgggttcgcctcgatgtaccggcggcctagggccgacgcgcggctttggcggtagatcccctcgagcagatcgtcgcttgccagcggccagtacggcagccagagctgctcaaattcgtcggcgacgtggctcacgcttggtagtagaccacgattaatcaccggtgtatggtccgacacgagctccaagtcagatatttcgctgaggggccaccccacaactgcacactcccccgctctcccgtcgagccctggtggtggaacaccagcgacagccgagcacccccaaccacctgtaccaaccaggaggaacacatgcgtcgtttcgaggacgtttccgggccgctgagagccgctgtggcggccgtacacgccgccttagacccgttagaccccctgccgcctgaatgcgcgggtacgagccacacagcgcccgaacttacggagctggtgggctcacctggctttatggcgtacgaatcggctgtgtgcgacctgttgggcgaggtgaggtacgcgctactcacgctggcaagggcgacacagccgccccaccgagcccgcacggccgcgcgcggtgtcaacaaccgggtgagtcgtgcacaccagcaggtgttcgaggcttggctcgaagtgcaggacatcgtggcgaacgccgcccgatgagccgcgccttacgctggctgccagccgttcgcgggctggttggtgcagcgcgtcgagcggttagaggccctgcggtgttccaccaccgcagggcctcgccctttttaaggctgaatttgcttgtctccgaatccaactggcttgtccaagggtgtatctacgcttaatccaaagttcaaacgaggggattacacatgaccaacttcgataacgttctcggctcgatcctgaatcgccccatcatccagccagaaagtgagggagccacggttgatgagagctttgttgtaggtggaccagttggtgattttgaacttttgctttgccacggaacggtctgcgttgtcgggaagatgcgtgatctgatccttcaactcagcaaaagttcgatttattcaacaaagccgccgtcccgtcaagtcagcgtaatgctctgccagtgttacaaccaattaaccaattctgattagaaaaactcatcgagcatcaaatgaaactgcaatttattcatatcaggattatcaataccatatttttgaaaaagccgtttctgtaatgaaggagaaaactcaccgaggcagttccataggatggcaagatcctggtatcggtctgcgattccgactcgtccaacatcaatacaacctattaatttcccctcgtcaaaaataaggttatcaagtgagaaatcaccatgagtgacgactgaatccggtgagaatggcaaaagcttatgcatttctttccagacttgttcaacaggccagccattacgctcgtcatcaaaatcactcgcatcaaccaaaccgttattcattcgtgattgcgcctgagcgagacgaaatacgcgatcgctgttaaaaggacaattacaaacaggaatcgaatgcaaccggcgcaggaacactgccagcgcatcaacaatattttcacctgaatcaggatattcttctaatacctggaatgctgttttcccggggatcgcagtggtgagtaaccatgcatcatcaggagtacggataaaatgcttgatggtcggaagaggcataaattccgtcagccagtttagtctgaccatctcatctgtaacatcattggcaacgctacctttgccatgtttcagaaacaactctggcgcatcgggcttcccatacaatcgatagattgtcgcacctgattgcccgacattatcgcgagcccatttatacccatataaatcagcatccatgttggaatttaatcgcggcctcgagcaagacgtttcccgttgaatatggctcataacaccccttgtattactgtttatgtaagcagacagttttattgttcatgatgatatatttttatcttgtgcaatgtaacatcagagattttgagacacaacgtggctttcccccccccccctatcattgcagcactggggccagatggtaagccctcccgtatcgtagttatctacacgacggggagtcaggcaactatggatgaacgaaatagacagatcgctgagataggtgcctcactgattaagcattggtaactgtcagaccaagtttactcatatatactttagattgatttaaaacttcatttttaatttaaaaggatctaggtgaagatcctttttgataatctcatgaccaaaatcccttaacgtgagttttcgttccactgagcgtcagaccccgtagaaaagatcaaaggatcttcttgagatcctttttttctgcgcgtaatctgctgcttgcaaacaaaaaaaccaccgctaccagcggtggtttgtttgccggatcaagagctaccaactctttttccgaaggtaactggcttcagcagagcgcagataccaaatactgtccttctagtgtagccgtagttaggccaccacttcaagaactctgtagcaccgcctacatacctcgctctgctaatcctgttaccagtggctgctgccagtggcgataagtcgtgtcttaccgggttggactcaagacgatagttaccggataaggcgcagcggtcgggctgaacggggggttcgtgcacacagcccagcttggagcgaacgacctacaccgaactgagatacctacagcgtgagctatgagaaagcgccacgcttcccgaagggagaaaggcggacaggtatccggtaagcggcagggtcggaacaggagagcgcacgagggagcttccagggggaaacgcctggtatctttatagtcctgtcgggtttcgccacctctgacttgagcgtcgatttttgtgatgctcgtcaggggggcggagcctatggaaaaacgccagcaacgcggcctttttacggttcctggccttttgctggccttttgctcacatgttctttcctgcgttatcccctgattctgtggataaccgtattaccgcctttgagtgagctgataccgctcgccgcagccgaacgaccgagcgcagcgagtcagtgagcgaggaagcggaaga